European Patent Application EP 4 148 126 A1, published March 15, 2023. Title: IMMUNOLOGICALLY CLOAKING ANTI-TUMOR ADENOVIRUS. Applicant: CURIGIN CO.,Ltd. The sequence listing filed with the application follows.

SEQUENCE LISTING (14 sequences)

SEQ ID NO: 1 - DNA, 195 bp, Artificial Sequence
  ABD
atgggctgtagcagccatgagcatgagcatgaggatgaagccgtcgacgcgaattcattagctgctgctaaagagacggctctgtatcatcttgacaggttgggagtagctgacgcttacaaggatctaatcgataaagccaaaactgttgaaggtgtaaaggcacggtattttgaaattttacatgcattaccc

SEQ ID NO: 2 - protein, 52 aa, Artificial Sequence
  ABD
GTIDEWLLKEAKEKAIEELKKAGITSDYYFDLINKAKTVEGVNALKDEILKA

SEQ ID NO: 3 - DNA, 2859 bp, Artificial Sequence
  Hexon
atggctaccccttcgatgatgccgcagtggtcttacatgcacatctcgggccaggacgcctcggagtacctgagccccgggctggtgcagtttgcccgcgccaccgagacgtacttcagcctgaataacaagtttagaaaccccacggtggcgcctacgcacgacgtgaccacagaccggtcccagcgtttgacgctgcggttcatccctgtggaccgtgaggatactgcgtactcgtacaaggcgcggttcaccctagctgtgggtgataaccgtgtgctggacatggcttccacgtactttgacatccgcggcgtgctggacaggggccctacttttaagccctactctggcactgcctacaacgccctggctcccaagggtgccccaaatccttgcgaatgggatgaagctgctactgctcttgaaataaacctagaagaagaggacgatgacaacgaagacgaagtagacgagcaagctgagcagcaaaaaactcacgtatttgggcaggcgccttattctggtataaatattacaaaggagggtattcaaataggtgtcgaaggtcaaacacctaaatatgccgataaaacatttcaacctgaacctcaaataggagaatctcagtggtacgaaacagaaattaatcatgcagctgggagagtcctaaaaaagactaccccaatgaaaccatgttacggttcatatgcaaaacccacaaatgaaaatggagggcaaggcattcttgtaaagcaacaaaatggaaagctagaaagtcaagtggaaatgcaatttttctcaactactgaggcagccgcaggcaatggtgataacttgactcctaaagtggtattgtacagtgaagatgtagatatagaaaccccagacactcatatttcttacatgcccactattaaggaaggtaactcacgagaactaatgggccaacaatctatgcccaacaggcctaattacattgcttttagggacaattttattggtctaatgtattacaacagcacgggtaatatgggtgttctggcgggccaagcatcgcagttgaatgctgttgtagatttgcaagacagaaacacagagctttcataccagcttttgcttgattccattggtgatagaaccaggtacttttctatgtggaatcaggctgttgacagctatgatccagatgttagaattattgaaaatcatggaactgaagatgaacttccaaattactgctttccactgggaggtgtgattaatacagagactcttaccaaggtaaaacctaaaacaggtcaggaaaatggatgggaaaaagatgctacagaattttcagataaaaatgaaataagagttggaaataattttgccatggaaatcaatctaaatgccaacctgtggagaaatttcctgtactccaacatagcgctgtatttgcccgacaagctaaagtacagtccttccaacgtaaaaatttctgataacccaaacacctacgactacatgaacaagcgagtggtggctcccgggctagtggactgctacattaaccttggagcacgctggtcccttgactatatggacaacgtcaacccatttaaccaccaccgcaatgctggcctgcgctaccgctcaatgttgctgggcaatggtcgctatgtgcccttccacatccaggtgcctcagaagttctttgccattaaaaacctccttctcctgccgggctcatacacctacgagtggaacttcaggaaggatgttaacatggttctgcagagctccctaggaaatgacctaagggttgacggagccagcattaagtttgatagcatttgcctttacgccaccttcttccccatggcccacaacaccgcctccacgcttgaggccatgcttagaaacgacaccaacgaccagtcctttaacgactatctctccgccgccaacatgctctaccctatacccgccaacgctaccaacgtgcccatatccatcccctcccgcaactgggcggctttccgcggctgggccttcacgcgccttaagactaaggaaaccccatcactgggctcgggctacgacccttattacacctactctggctctataccctacctagatggaaccttttacctcaaccacacctttaagaaggtggccattacctttgactcttctgtcagctggcctggcaatgaccgcctgcttacccccaacgagtttgaaattaagcgctcagttgacggggagggttacaacgttgcccagtgtaacatgaccaaagactggttcctggtacaaatgctagctaactataacattggctaccagggcttctatatcccagagagctacaaggaccgcatgtactccttctttagaaacttccagcccatgagccgtcaggtggtggatgatactaaatacaaggactaccaacaggtgggcatcctacaccaacacaacaactctggatttgttggctaccttgcccccaccatgcgcgaaggacaggcctaccctgctaacttcccctatccgcttataggcaagaccgcagttgacagcattacccagaaaaagtttctttgcgatcgcaccctttggcgcatcccattctccagtaactttatgtccatgggcgcactcacagacctgggccaaaaccttctctacgccaactccgcccacgcgctagacatgacttttgaggtggatcccatggacgagcccacccttctttatgttttgtttgaagtctttgacgtggtccgtgtgcaccagccgcaccgcggcgtcatcgaaaccgtgtacctgcgcacgcccttctcggccggcaacgccacaacataa

SEQ ID NO: 4 - DNA, 3762 bp, Artificial Sequence
  hTERT-E1A-IRES-E1B
tggcccctccctcgggttaccccacagcctaggccgattcgacctctctccgctggggccctcgctggcgtccctgcaccctgggagcgcgagcggcgcgcgggcggggaagcgcggcccagacccccgggtccgcccggagcagctgcgctgtcggggccaggccgggctcccagtggattcgcgggcacagacgcccaggaccgcgctccccacgtggcggagggactggggacccgggcacccgtcctgccccttcaccttccagctccgcctcctccgcgcggaccccgccccgtcccgacccctcccgggtccccggcccagccccctccgggccctcccagcccctccccttcctttccgcggccccgccctctcctcgcggcgcgagtttcaggcagcgctgcgtcctgctgcgcacgtgggaagccctggccccggccacccccgcgactagtacaccgggactgaaaatgagacatattatctgccacggaggtgttattaccgaagaaatggccgccagtcttttggaccagctgatcgaagaggtactggctgataatcttccacctcctagccattttgaaccacctacccttcacgaactgtatgatttagacgtgacggcccccgaagatcccaacgaggaggcggtttcgcagatttttcccgactctgtaatgttggcggtgcaggaagggattgacttactcacttttccgccggcgcccggttctccggagccgcctcacctttcccggcagcccgagcagccggagcagagagccttgggtccggtttctatgccaaaccttgtaccggaggtgatcgatcttacctgccacgaggctggctttccacccagtgacgacgaggatgaagagggtgaggagtttgtgttagattatgtggagcaccccgggcacggttgcaggtcttgtcattatcaccggaggaatacgggggacccagatattatgtgttcgctttgctatatgaggacctgtggcatgtttgtctacagtcctgtgtctgaacctgagcctgagcccgagccagaaccggagcctgcaagacctacccgccgtcctaaaatggcgcctgctatcctgagacgcccgacatcacctgtgtctagagaatgcaatagtagtacggatagctgtgactccggtccttctaacacacctcctgagatacacccggtggtcccgctgtgccccattaaaccagttgccgtgagagttggtgggcgtcgccaggctgtggaatgtatcgaggacttgcttaacgagcctgggcaacctttggacttgagctgtaaacgccccaggccataaggtgtaaacctgtgacccctctccctcccccccctaacgttactggccgaagccgcttggaataaggccggtgtgcgtttgtctatatgttattttccaccatattgccgtcttttggcaatgtgagggcccggaaacctggccctgtcttcttgacgagcattcctaggggtctttcccctctcgccaaaggaatgcaaggtctgttgaatgtcgtgaaggaagcagttcctctggaagcttcttgaagacaaacaacgtctgtagcgaccctttgcaggcagcggaaccccccacctggcgacaggtgcctctgcggccaaaagccacgtgtataagatacacctgcaaaggcggcacaaccccagtgccacgttgtgagttggatagttgtggaaagagtcaaatggctctcctcaagcgtattcaacaaggggctgaaggatgcccagaaggtaccccattgtatgggatctgatctggggcctcggtgcacatgctttacatgtgtttagtcgaggttaaaaaaacgtctaggccccccgaaccacggggacgtggttttcctttgaaaaacacgatgataagcttgccacaacccgggatcctctagagtcgacatggaggcttgggagtgtttggaagatttttctgctgtgcgtaacttgctggaacagagctctaacagtacctcttggttttggaggtttctgtggggctcatcccaggcaaagttagtctgcagaattaaggaggattacaagtgggaatttgaagagcttttgaaatcctgtggtgagctgtttgattctttgaatctgggtcaccaggcgcttttccaagagaaggtcatcaagactttggatttttccacaccggggcgcgctgcggctgctgttgcttttttgagttttataaaggataaatggagcgaagaaacccatctgagcggggggtacctgctggattttctggccatgcatctgtggagagcggttgtgagacacaagaatcgcctgctactgttgtcttccgtccgcccggcgataataccgacggaggagcagcagcagcagcaggaggaagccaggcggcggcggcaggagcagagcccatggaacccgagagccggcctggaccctcgggaatgaatgttgtacaggtggctgaactgtatccagaactgagacgcattttgacaattacagaggatgggcaggggctaaagggggtaaagagggagcggggggcttgtgaggctacagaggaggctaggaatctagcttttagcttaatgaccagacaccgtcctgagtgtattacttttcaacagatcaaggataattgcgctaatgagcttgatctgctggcgcagaagtattccatagagcagctgaccacttactggctgcagccaggggatgattttgaggaggctattagggtatatgcaaaggtggcacttaggccagattgcaagtacaagatcagcaaacttgtaaatatcaggaattgttgctacatttctgggaacggggccgaggtggagatagatacggaggatagggtggcctttagatgtagcatgataaatatgtggccgggggtgcttggcatggacggggtggttattatgaatgtaaggtttactggccccaattttagcggtacggttttcctggccaataccaaccttatcctacacggtgtaagcttctatgggtttaacaatacctgtgtggaagcctggaccgatgtaagggttcggggctgtgccttttactgctgctggaagggggtggtgtgtcgccccaaaagcagggcttcaattaagaaatgcctctttgaaaggtgtaccttgggtatcctgtctgagggtaactccagggtgcgccacaatgtggcctccgactgtggttgcttcatgctagtgaaaagcgtggctgtgattaagcataacatggtatgtggcaactgcgaggacagggcctctcagatgctgacctgctcggacggcaactgtcacctgctgaagaccattcacgtagccagccactctcgcaaggcctggccagtgtttgagcataacatactgacccgctgttccttgcatttgggtaacaggaggggggtgttcctaccttaccaatgcaatttgagtcacactaagatattgcttgagcccgagagcatgtccaaggtgaacctgaacggggtgtttgacatgaccatgaagatctggaaggtgctgaggtacgatgagacccgcaccaggtgcagaccctgcgagtgtggcggtaaacatattaggaaccagcctgtgatgctggatgtgaccgaggagctgaggcccgatcacttggtgctggcctgcacccgcgctgagtttggctctagcgatgaagatacagattga

SEQ ID NO: 5 - DNA, 1296 bp, Artificial Sequence
  CMVpromoter-Dasher GFP
cgttacataacttacggtaaatggcccgcctggctgaccgcccaacgacccccgcccattgacgtcaataatgacgtatgttcccatagtaacgccaatagggactttccattgacgtcaatgggtggagtatttacggtaaactgcccacttggcagtacatcaagtgtatcatatgccaagtacgccccctattgacgtcaatgacggtaaatggcccgcctggcattatgcccagtacatgaccttatgggactttcctacttggcagtacatctacgtattagtcatcgctattaccatggtgatgcggttttggcagtacatcaatgggcgtggatagcggtttgactcacggggatttccaagtctccaccccattgacgtcaatgggagtttgttttggcaccaaaatcaacgggactttccaaaatgtcgtaacaactccgccccattgacgcaaatgggcggtaggcgtgtacggtgggaggtctatataagcagagctcgtttagtgaaccgtcagatcgcctggagacgccatccacgctgttttgacctccatagaagacaccggccgccaccatgactgccctgaccgaaggtgctaagctgtttgagaaggagattccgtacatcaccgagctggaaggggacgtcgaaggaatgaagttcatcatcaagggagaaggaaccggggacgctacgactggaaccattaaggccaagtatatctgtaccactggagatctgccagtgccttgggccacccttgtgtcaaccctctcgtatggagtgcagtgttttgctaagtaccctagccacattaaggacttcttcaaatccgccatgccggaaggttatacccaagagcgcaccatttcttttgagggagatggagtgtacaagacccgcgcgatggtcacctatgagaggggatctatctacaaccgggtgactctgactggagaaaactttaagaaggacgggcatattcttcggaagaatgtcgccttccagtgccctcccagcatcctttacattctccccgacactgtgaacaacggaatccgcgtggagttcaatcaagcctacgacatcgagggggtgacggagaagctggtgaccaagtgtagccagatgaatcggccactggccggttcagcggctgtccacattccgcgctaccatcatatcacttatcacactaagctctccaaagaccgcgatgagaggagagatcacatgtgcctggtggaagtggtcaaggccgtcgatctcgatacctatcagtaa

SEQ ID NO: 6 - DNA, 3054 bp, Artificial Sequence
  Hexon-ABD-Hexon
atggctaccccttcgatgatgccgcagtggtcttacatgcacatctcgggccaggacgcctcggagtacctgagccccgggctggtgcagtttgcccgcgccaccgagacgtacttcagcctgaataacaagtttagaaaccccacggtggcgcctacgcacgacgtgaccacagaccggtcccagcgtttgacgctgcggttcatccctgtggaccgtgaggatactgcgtactcgtacaaggcgcggttcaccctagctgtgggtgataaccgtgtgctggacatggcttccacgtactttgacatccgcggcgtgctggacaggggccctacttttaagccctactctggcactgcctacaacgccctggctcccaagggtgccccaaatccttgcgaatgggatgaagctgctactgctcttgaaataaacctagaagaagaggacgatgacaacgaaatgggctgtagcagccatgagcatgagcatgaggatgaagccgtcgacgcgaattcattagctgctgctaaagagacggctctgtatcatcttgacaggttgggagtagctgacgcttacaaggatctaatcgataaagccaaaactgttgaaggtgtaaaggcacggtattttgaaattttacatgcattacccgacgaagtagacgagcaagctgagcagcaaaaaactcacgtatttgggcaggcgccttattctggtataaatattacaaaggagggtattcaaataggtgtcgaaggtcaaacacctaaatatgccgataaaacatttcaacctgaacctcaaataggagaatctcagtggtacgaaacagaaattaatcatgcagctgggagagtcctaaaaaagactaccccaatgaaaccatgttacggttcatatgcaaaacccacaaatgaaaatggagggcaaggcattcttgtaaagcaacaaaatggaaagctagaaagtcaagtggaaatgcaatttttctcaactactgaggcagccgcaggcaatggtgataacttgactcctaaagtggtattgtacagtgaagatgtagatatagaaaccccagacactcatatttcttacatgcccactattaaggaaggtaactcacgagaactaatgggccaacaatctatgcccaacaggcctaattacattgcttttagggacaattttattggtctaatgtattacaacagcacgggtaatatgggtgttctggcgggccaagcatcgcagttgaatgctgttgtagatttgcaagacagaaacacagagctttcataccagcttttgcttgattccattggtgatagaaccaggtacttttctatgtggaatcaggctgttgacagctatgatccagatgttagaattattgaaaatcatggaactgaagatgaacttccaaattactgctttccactgggaggtgtgattaatacagagactcttaccaaggtaaaacctaaaacaggtcaggaaaatggatgggaaaaagatgctacagaattttcagataaaaatgaaataagagttggaaataattttgccatggaaatcaatctaaatgccaacctgtggagaaatttcctgtactccaacatagcgctgtatttgcccgacaagctaaagtacagtccttccaacgtaaaaatttctgataacccaaacacctacgactacatgaacaagcgagtggtggctcccgggctagtggactgctacattaaccttggagcacgctggtcccttgactatatggacaacgtcaacccatttaaccaccaccgcaatgctggcctgcgctaccgctcaatgttgctgggcaatggtcgctatgtgcccttccacatccaggtgcctcagaagttctttgccattaaaaacctccttctcctgccgggctcatacacctacgagtggaacttcaggaaggatgttaacatggttctgcagagctccctaggaaatgacctaagggttgacggagccagcattaagtttgatagcatttgcctttacgccaccttcttccccatggcccacaacaccgcctccacgcttgaggccatgcttagaaacgacaccaacgaccagtcctttaacgactatctctccgccgccaacatgctctaccctatacccgccaacgctaccaacgtgcccatatccatcccctcccgcaactgggcggctttccgcggctgggccttcacgcgccttaagactaaggaaaccccatcactgggctcgggctacgacccttattacacctactctggctctataccctacctagatggaaccttttacctcaaccacacctttaagaaggtggccattacctttgactcttctgtcagctggcctggcaatgaccgcctgcttacccccaacgagtttgaaattaagcgctcagttgacggggagggttacaacgttgcccagtgtaacatgaccaaagactggttcctggtacaaatgctagctaactataacattggctaccagggcttctatatcccagagagctacaaggaccgcatgtactccttctttagaaacttccagcccatgagccgtcaggtggtggatgatactaaatacaaggactaccaacaggtgggcatcctacaccaacacaacaactctggatttgttggctaccttgcccccaccatgcgcgaaggacaggcctaccctgctaacttcccctatccgcttataggcaagaccgcagttgacagcattacccagaaaaagtttctttgcgatcgcaccctttggcgcatcccattctccagtaactttatgtccatgggcgcactcacagacctgggccaaaaccttctctacgccaactccgcccacgcgctagacatgacttttgaggtggatcccatggacgagcccacccttctttatgttttgtttgaagtctttgacgtggtccgtgtgcaccagccgcaccgcggcgtcatcgaaaccgtgtacctgcgcacgcccttctcggccggcaacgccacaacataa

SEQ ID NO: 7 - DNA, 455 bp, Artificial Sequence
  hTERT promoter
tggcccctccctcgggttaccccacagcctaggccgattcgacctctctccgctggggccctcgctggcgtccctgcaccctgggagcgcgagcggcgcgcgggcggggaagcgcggcccagacccccgggtccgcccggagcagctgcgctgtcggggccaggccgggctcccagtggattcgcgggcacagacgcccaggaccgcgctccccacgtggcggagggactggggacccgggcacccgtcctgccccttcaccttccagctccgcctcctccgcgcggaccccgccccgtcccgacccctcccgggtccccggcccagccccctccgggccctcccagcccctccccttcctttccgcggccccgccctctcctcgcggcgcgagtttcaggcagcgctgcgtcctgctgcgcacgtgggaagccctggccccggccacccccgcg

SEQ ID NO: 8 - DNA, 900 bp, Artificial Sequence
  E1A gene
acaccgggactgaaaatgagacatattatctgccacggaggtgttattaccgaagaaatggccgccagtcttttggaccagctgatcgaagaggtactggctgataatcttccacctcctagccattttgaaccacctacccttcacgaactgtatgatttagacgtgacggcccccgaagatcccaacgaggaggcggtttcgcagatttttcccgactctgtaatgttggcggtgcaggaagggattgacttactcacttttccgccggcgcccggttctccggagccgcctcacctttcccggcagcccgagcagccggagcagagagccttgggtccggtttctatgccaaaccttgtaccggaggtgatcgatcttacctgccacgaggctggctttccacccagtgacgacgaggatgaagagggtgaggagtttgtgttagattatgtggagcaccccgggcacggttgcaggtcttgtcattatcaccggaggaatacgggggacccagatattatgtgttcgctttgctatatgaggacctgtggcatgtttgtctacagtcctgtgtctgaacctgagcctgagcccgagccagaaccggagcctgcaagacctacccgccgtcctaaaatggcgcctgctatcctgagacgcccgacatcacctgtgtctagagaatgcaatagtagtacggatagctgtgactccggtccttctaacacacctcctgagatacacccggtggtcccgctgtgccccattaaaccagttgccgtgagagttggtgggcgtcgccaggctgtggaatgtatcgaggacttgcttaacgagcctgggcaacctttggacttgagctgtaaacgccccaggccataaggtgtaaacctgtga

SEQ ID NO: 9 - DNA, 1797 bp, Artificial Sequence
  E1B gene
catggaggcttgggagtgtttggaagatttttctgctgtgcgtaacttgctggaacagagctctaacagtacctcttggttttggaggtttctgtggggctcatcccaggcaaagttagtctgcagaattaaggaggattacaagtgggaatttgaagagcttttgaaatcctgtggtgagctgtttgattctttgaatctgggtcaccaggcgcttttccaagagaaggtcatcaagactttggatttttccacaccggggcgcgctgcggctgctgttgcttttttgagttttataaaggataaatggagcgaagaaacccatctgagcggggggtacctgctggattttctggccatgcatctgtggagagcggttgtgagacacaagaatcgcctgctactgttgtcttccgtccgcccggcgataataccgacggaggagcagcagcagcagcaggaggaagccaggcggcggcggcaggagcagagcccatggaacccgagagccggcctggaccctcgggaatgaatgttgtacaggtggctgaactgtatccagaactgagacgcattttgacaattacagaggatgggcaggggctaaagggggtaaagagggagcggggggcttgtgaggctacagaggaggctaggaatctagcttttagcttaatgaccagacaccgtcctgagtgtattacttttcaacagatcaaggataattgcgctaatgagcttgatctgctggcgcagaagtattccatagagcagctgaccacttactggctgcagccaggggatgattttgaggaggctattagggtatatgcaaaggtggcacttaggccagattgcaagtacaagatcagcaaacttgtaaatatcaggaattgttgctacatttctgggaacggggccgaggtggagatagatacggaggatagggtggcctttagatgtagcatgataaatatgtggccgggggtgcttggcatggacggggtggttattatgaatgtaaggtttactggccccaattttagcggtacggttttcctggccaataccaaccttatcctacacggtgtaagcttctatgggtttaacaatacctgtgtggaagcctggaccgatgtaagggttcggggctgtgccttttactgctgctggaagggggtggtgtgtcgccccaaaagcagggcttcaattaagaaatgcctctttgaaaggtgtaccttgggtatcctgtctgagggtaactccagggtgcgccacaatgtggcctccgactgtggttgcttcatgctagtgaaaagcgtggctgtgattaagcataacatggtatgtggcaactgcgaggacagggcctctcagatgctgacctgctcggacggcaactgtcacctgctgaagaccattcacgtagccagccactctcgcaaggcctggccagtgtttgagcataacatactgacccgctgttccttgcatttgggtaacaggaggggggtgttcctaccttaccaatgcaatttgagtcacactaagatattgcttgagcccgagagcatgtccaaggtgaacctgaacggggtgtttgacatgaccatgaagatctggaaggtgctgaggtacgatgagacccgcaccaggtgcagaccctgcgagtgtggcggtaaacatattaggaaccagcctgtgatgctggatgtgaccgaggagctgaggcccgatcacttggtgctggcctgcacccgcgctgagtttggctctagcgatgaagatacagattga

SEQ ID NO: 10 - DNA, 572 bp, Artificial Sequence
  IRES
cccctctccctcccccccctaacgttactggccgaagccgcttggaataaggccggtgtgcgtttgtctatatgttattttccaccatattgccgtcttttggcaatgtgagggcccggaaacctggccctgtcttcttgacgagcattcctaggggtctttcccctctcgccaaaggaatgcaaggtctgttgaatgtcgtgaaggaagcagttcctctggaagcttcttgaagacaaacaacgtctgtagcgaccctttgcaggcagcggaaccccccacctggcgacaggtgcctctgcggccaaaagccacgtgtataagatacacctgcaaaggcggcacaaccccagtgccacgttgtgagttggatagttgtggaaagagtcaaatggctctcctcaagcgtattcaacaaggggctgaaggatgcccagaaggtaccccattgtatgggatctgatctggggcctcggtgcacatgctttacatgtgtttagtcgaggttaaaaaaacgtctaggccccccgaaccacggggacgtggttttcctttgaaaaacacgatgataa

SEQ ID NO: 11 - DNA, 508 bp, Artificial Sequence
  CMV promoter
cgttacataacttacggtaaatggcccgcctggctgaccgcccaacgacccccgcccattgacgtcaataatgacgtatgttcccatagtaacgccaatagggactttccattgacgtcaatgggtggagtatttacggtaaactgcccacttggcagtacatcaagtgtatcatatgccaagtacgccccctattgacgtcaatgacggtaaatggcccgcctggcattatgcccagtacatgaccttatgggactttcctacttggcagtacatctacgtattagtcatcgctattaccatggtgatgcggttttggcagtacatcaatgggcgtggatagcggtttgactcacggggatttccaagtctccaccccattgacgtcaatgggagtttgttttggcaccaaaatcaacgggactttccaaaatgtcgtaacaactccgccccattgacgcaaatgggcggtaggcgtgtacggtgggaggtctatataagcagagct

SEQ ID NO: 12 - DNA, 711 bp, Artificial Sequence
  GFP
atgactgccctgaccgaaggtgctaagctgtttgagaaggagattccgtacatcaccgagctggaaggggacgtcgaaggaatgaagttcatcatcaagggagaaggaaccggggacgctacgactggaaccattaaggccaagtatatctgtaccactggagatctgccagtgccttgggccacccttgtgtcaaccctctcgtatggagtgcagtgttttgctaagtaccctagccacattaaggacttcttcaaatccgccatgccggaaggttatacccaagagcgcaccatttcttttgagggagatggagtgtacaagacccgcgcgatggtcacctatgagaggggatctatctacaaccgggtgactctgactggagaaaactttaagaaggacgggcatattcttcggaagaatgtcgccttccagtgccctcccagcatcctttacattctccccgacactgtgaacaacggaatccgcgtggagttcaatcaagcctacgacatcgagggggtgacggagaagctggtgaccaagtgtagccagatgaatcggccactggccggttcagcggctgtccacattccgcgctaccatcatatcacttatcacactaagctctccaaagaccgcgatgagaggagagatcacatgtgcctggtggaagtggtcaaggccgtcgatctcgatacctatcagtaa

SEQ ID NO: 13 - DNA, 420 bp, Artificial Sequence
  pIX
atgagcaccaactcgtttgatggaagcattgtgagctcatatttgacaacgcgcatgcccccatgggccggggtgcgtcagaatgtgatgggctccagcattgatggtcgccccgtcctgcccgcaaactctactaccttgacctacgagaccgtgtctggaacgccgttggagactgcagcctccgccgccgcttcagccgctgcagccaccgcccgcgggattgtgactgactttgctttcctgagcccgcttgcaagcagtgcagcttcccgttcatccgcccgcgatgacaagttgacggctcttttggcacaattggattctttgacccgggaacttaatgtcgtttctcagcagctgttggatctgcgccagcaggtttctgccctgaaggcttcctcccctcccaatgcggtt

SEQ ID NO: 14 - DNA, 618 bp, Artificial Sequence
  pIX-ABD
atgagcaccaactcgtttgatggaagcattgtgagctcatatttgacaacgcgcatgcccccatgggccggggtgcgtcagaatgtgatgggctccagcattgatggtcgccccgtcctgcccgcaaactctactaccttgacctacgagaccgtgtctggaacgccgttggagactgcagcctccgccgccgcttcagccgctgcagccaccgcccgcgggattgtgactgactttgctttcctgagcccgcttgcaagcagtgcagcttcccgttcatccgcccgcgatgacaagttgacggctcttttggcacaattggattctttgacccgggaacttaatgtcgtttctcagcagctgttggatctgcgccagcaggtttctgccctgaaggcttcctcccctcccaatgcggttatgggctgtagcagccatgagcatgagcatgaggatgaagccgtcgacgcgaattcattagctgctgctaaagagacggctctgtatcatcttgacaggttgggagtagctgacgcttacaaggatctaatcgataaagccaaaactgttgaaggtgtaaaggcacggtattttgaaattttacatgcattaccctaa